European Patent Application EP 4 470 568 A1, published December 4, 2024. Title: PHARMACEUTICAL COMPOSITION COMPRISING ANTI-CD79B ANTIBODY-DRUG CONJUGATE AND USE THEREOF. Applicant: Shanghai MabGen Biotech Ltd. The sequence listing filed with the application follows.

SEQUENCE LISTING (15 sequences)

SEQ ID NO: 1 - protein, 117 aa, synthetic construct
  source 1..117: note = mAb015 VH
QVQLQQSGAELARPGASVKLSCKASGSSFTSYGINWVKQRTGQGLEWIGEIFPRSGNTYYNEKFEGKATLTADKSSSTAYMELRSLTSEDSAVYFCAKGDLGDFDYWGQGTTLTVSS

SEQ ID NO: 2 - protein, 112 aa, synthetic construct
  source 1..112: note = mAb015 VL
DFLMTQTPLSLPVRLGDQASISCRSSQSIVHSDGNTYFEWYLQKPGQSPKLLIYKVSNRFSGVPDRFSGSGSGTDFTLKISRVEAEDLGVYYCFQGSHVPWTFGGGTKLEIK

SEQ ID NO: 3 - protein, 117 aa, synthetic construct
  source 1..117: note = hAb015-10 VH
EVQLVQSGAEVKKPGSSVKVSCKASGSSFSSYGINWVKQAPGQGLEWIGEIFPRSGNTYYNEKFEGRATLTADKSTSTAYMELRSLRSEDTAVYYCAKGDLGDFDYWGQGTTVTVSS

SEQ ID NO: 4 - protein, 112 aa, synthetic construct
  source 1..112: note = hAb015-10 VL
DFVMTQTPLSLPVTPGEPASISCRSSQSIVHSDGNTYFEWYLQKPGQSPKLLIYKVSNRFSGVPDRFSGSGSGTDFTLKISRVEAEDVGVYYCFQGSHVPWTFGGGTKVEIK

SEQ ID NO: 5 - protein, 7 aa, synthetic construct
  source 1..7: note = HCDR1 (mAb015 )
GSSFTSY

SEQ ID NO: 6 - protein, 6 aa, synthetic construct
  source 1..6: note = HCDR2
FPRSGN

SEQ ID NO: 7 - protein, 8 aa, synthetic construct
  source 1..8: note = HCDR3
GDLGDFDY

SEQ ID NO: 8 - protein, 16 aa, synthetic construct
  source 1..16: note = LCDR1
RSSQSIVHSDGNTYFE

SEQ ID NO: 9 - protein, 7 aa, synthetic construct
  source 1..7: note = LCDR2
KVSNRFS

SEQ ID NO: 10 - protein, 9 aa, synthetic construct
  source 1..9: note = LCDR3
FQGSHVPWT

SEQ ID NO: 11 - protein, 7 aa, synthetic construct
  source 1..7: note = HCDR1 (hAb015-10)
GSSFSSY

SEQ ID NO: 12 - protein, 447 aa, synthetic construct
  source 1..447: note = hAb015-10 heavy chain
EVQLVQSGAEVKKPGSSVKVSCKASGSSFSSYGINWVKQAPGQGLEWIGEIFPRSGNTYYNEKFEGRATLTADKSTSTAYMELRSLRSEDTAVYYCAKGDLGDFDYWGQGTTVTVSSASTKGPSVFPLAPSSKSTSGGTAALGCLVKDYFPEPVTVSWNSGALTSGVHTFPAVLQSSGLYSLSSVVTVPSSSLGTQTYICNVNHKPSNTKVDKKVEPKSCDKTHTCPPCPAPELLGGPSVFLFPPKPKDTLMISRTPEVTCVVVDVSHEDPEVKFNWYVDGVEVHNAKTKPREEQYNSTYRVVSVLTVLHQDWLNGKEYKCKVSNKALPAPIEKTISKAKGQPREPQVYTLPPSREEMTKNQVSLTCLVKGFYPSDIAVEWESNGQPENNYKTTPPVLDSDGSFFLYSKLTVDKSRWQQGNVFSCSVMHEALHNHYTQKSLSLSPGK

SEQ ID NO: 13 - protein, 219 aa, synthetic construct
  source 1..219: note = hAb015-10 light chain
DFVMTQTPLSLPVTPGEPASISCRSSQSIVHSDGNTYFEWYLQKPGQSPKLLIYKVSNRFSGVPDRFSGSGSGTDFTLKISRVEAEDVGVYYCFQGSHVPWTFGGGTKVEIKRTVAAPSVFIFPPSDEQLKSGTASVVCLLNNFYPREAKVQWKVDNALQSGNSQESVTEQDSKDSTYSLSSTLTLSKADYEKHKVYACEVTHQGLSSPVTKSFNRGEC

SEQ ID NO: 14 - protein, 447 aa, synthetic construct
  source 1..447: note = SN8 heavy chain
EVQLVESGGGLVQPGGSLRLSCAASGYTFSSYWIEWVRQAPGKGLEWIGEILPGGGDTNYNEIFKGRATFSADTSKNTAYLQMNSLRAEDTAVYYCTRRVPIRLDYWGQGTLVTVSSASTKGPSVFPLAPSSKSTSGGTAALGCLVKDYFPEPVTVSWNSGALTSGVHTFPAVLQSSGLYSLSSVVTVPSSSLGTQTYICNVNHKPSNTKVDKKVEPKSCDKTHTCPPCPAPELLGGPSVFLFPPKPKDTLMISRTPEVTCVVVDVSHEDPEVKFNWYVDGVEVHNAKTKPREEQYNSTYRVVSVLTVLHQDWLNGKEYKCKVSNKALPAPIEKTISKAKGQPREPQVYTLPPSREEMTKNQVSLTCLVKGFYPSDIAVEWESNGQPENNYKTTPPVLDSDGSFFLYSKLTVDKSRWQQGNVFSCSVMHEALHNHYTQKSLSLSPGK

SEQ ID NO: 15 - protein, 218 aa, synthetic construct
  source 1..218: note = SN8 light chain
DIQLTQSPSSLSASVGDRVTITCKASQSVDYEGDSFLNWYQQKPGKAPKLLIYAASNLESGVPSRFSGSGSGTDFTLTISSLQPEDFATYYCQQSNEDPLTFGQGTKVEIKRTVAAPSVFIFPPSDEQLKSGTASVVCLLNNFYPREAKVQWKVDNALQSGNSQESVTEQDSKDSTYSLSSTLTLSKADYEKHKVYACEVTHQGLSSPVTKSFNRGEC